European Patent Application EP 4 509 140 A1, published February 19, 2025. Title: CONJUGATE, PHARMACEUTICAL COMPOSITION COMPRISING SAME, METHOD FOR PREPARING SAME, AND USE THEREOF. Applicant: SUZHOU RIBO LIFE SCIENCE CO., LTD. The sequence listing filed with the application follows.

SEQUENCE LISTING (57 sequences)

SEQ ID NO: 1 - RNA, 21 nt, synthetic construct
  source 1..21: mol_type = other RNA
ctgcttcagacgtgttagctt

SEQ ID NO: 2 - RNA, 22 nt, synthetic construct
  source 1..22: mol_type = other RNA
ctgagttcagacgtgttgctct

SEQ ID NO: 3 - RNA, 32 nt, synthetic construct
  source 1..32: mol_type = other RNA
tctatggctgccgatctggtctccatgtacgt

SEQ ID NO: 4 - RNA, 21 nt, synthetic construct
  source 1..21: mol_type = other RNA
  misc_feature 1: note = is CU, UC or AC
  misc_feature 13: note = is U, C or G or a motif consisting of two of U, C or G
  misc_feature 16: note = is U, CU or UU
  misc_feature 21: note = is U, UU or UUN8, N8 is a motif consisting of 1-15 nucleotides
nggagttcannnntgngctcn

SEQ ID NO: 5 - RNA, 24 nt, synthetic construct
  source 1..24: mol_type = other RNA
ctggagttcagacgtgttgctctt

SEQ ID NO: 6 - RNA, 24 nt, synthetic construct
  source 1..24: mol_type = other RNA
ctggagttcagacgttgtgctctt

SEQ ID NO: 7 - RNA, 24 nt, synthetic construct
  source 1..24: mol_type = other RNA
ctggagttcagaccgtgtgctctt

SEQ ID NO: 8 - RNA, 23 nt, synthetic construct
  source 1..23: mol_type = other RNA
ctggagttcagacgtgttgctct

SEQ ID NO: 9 - RNA, 24 nt, synthetic construct
  source 1..24: mol_type = other RNA
acggagttcagacgtgttgctctt

SEQ ID NO: 10 - RNA, 24 nt, synthetic construct
  source 1..24: mol_type = other RNA
ctggagttcactactgttgctctt

SEQ ID NO: 11 - RNA, 24 nt, synthetic construct
  source 1..24: mol_type = other RNA
ctggagttcagttgtgttgctctt

SEQ ID NO: 12 - RNA, 32 nt, synthetic construct
  source 1..32: mol_type = other RNA
ctggagttcagacgtgttgctcttccgatctc

SEQ ID NO: 13 - RNA, 32 nt, synthetic construct
  source 1..32: mol_type = other RNA
ctggagttcagacgttgtgctcttccgatctc

SEQ ID NO: 14 - RNA, 32 nt, synthetic construct
  source 1..32: mol_type = other RNA
ctggagttcagaccgtgtgctcttccgatctc

SEQ ID NO: 15 - RNA, 32 nt, synthetic construct; identical to SEQ ID NO: 12
  source 1..32: mol_type = other RNA

SEQ ID NO: 16 - RNA, 24 nt, synthetic construct
  source 1..24: mol_type = other RNA
ctggagttcagacgtgttgctctt

SEQ ID NO: 17 - RNA, 32 nt, synthetic construct; identical to SEQ ID NO: 13
  source 1..32: mol_type = other RNA

SEQ ID NO: 18 - RNA, 24 nt, synthetic construct
  source 1..24: mol_type = other RNA
ctggagttcagacgttgtgctctt

SEQ ID NO: 19 - RNA, 32 nt, synthetic construct; identical to SEQ ID NO: 14
  source 1..32: mol_type = other RNA

SEQ ID NO: 20 - RNA, 24 nt, synthetic construct
  source 1..24: mol_type = other RNA
ctggagttcagaccgtgtgctctt

SEQ ID NO: 21 - RNA, 32 nt, synthetic construct; identical to SEQ ID NO: 12
  source 1..32: mol_type = other RNA

SEQ ID NO: 22 - RNA, 24 nt, synthetic construct
  source 1..24: mol_type = other RNA
ctggagttcagacgtgttgctctt

SEQ ID NO: 23 - RNA, 32 nt, synthetic construct; identical to SEQ ID NO: 13
  source 1..32: mol_type = other RNA

SEQ ID NO: 24 - RNA, 24 nt, synthetic construct
  source 1..24: mol_type = other RNA
ctggagttcagacgttgtgctctt

SEQ ID NO: 25 - RNA, 32 nt, synthetic construct; identical to SEQ ID NO: 14
  source 1..32: mol_type = other RNA

SEQ ID NO: 26 - RNA, 24 nt, synthetic construct
  source 1..24: mol_type = other RNA
ctggagttcagaccgtgtgctctt

SEQ ID NO: 27 - RNA, 23 nt, synthetic construct
  source 1..23: mol_type = other RNA
ctggagttcagacgtgttgctct

SEQ ID NO: 28 - RNA, 22 nt, synthetic construct
  source 1..22: mol_type = other RNA
ctgagttcagacgtgttgctct

SEQ ID NO: 29 - RNA, 21 nt, synthetic construct
  source 1..21: mol_type = other RNA
ctgcttcagacgtgttagctt

SEQ ID NO: 30 - RNA, 24 nt, synthetic construct
  source 1..24: mol_type = other RNA
acggagttcagacgtgttgctctt

SEQ ID NO: 31 - RNA, 24 nt, synthetic construct
  source 1..24: mol_type = other RNA
ctggagttcactactgttgctctt

SEQ ID NO: 32 - RNA, 24 nt, synthetic construct
  source 1..24: mol_type = other RNA
ctggagttcagttgtgttgctctt

SEQ ID NO: 33 - RNA, 32 nt, synthetic construct; identical to SEQ ID NO: 3
  source 1..32: mol_type = other RNA

SEQ ID NO: 34 - RNA, 32 nt, synthetic construct; identical to SEQ ID NO: 12
  source 1..32: mol_type = other RNA

SEQ ID NO: 35 - RNA, 24 nt, synthetic construct
  source 1..24: mol_type = other RNA
ctggagttcagacgtgttgctctt

SEQ ID NO: 36 - RNA, 32 nt, synthetic construct; identical to SEQ ID NO: 13
  source 1..32: mol_type = other RNA

SEQ ID NO: 37 - RNA, 24 nt, synthetic construct
  source 1..24: mol_type = other RNA
ctggagttcagacgttgtgctctt

SEQ ID NO: 38 - RNA, 32 nt, synthetic construct; identical to SEQ ID NO: 14
  source 1..32: mol_type = other RNA

SEQ ID NO: 39 - RNA, 24 nt, synthetic construct
  source 1..24: mol_type = other RNA
ctggagttcagaccgtgtgctctt

SEQ ID NO: 40 - RNA, 17 nt, synthetic construct
  source 1..17: mol_type = other RNA
gtacattctagatagcc

SEQ ID NO: 41 - RNA, 17 nt, synthetic construct
  source 1..17: mol_type = other RNA
ggctatctagaatgtac

SEQ ID NO: 42 - RNA, 17 nt, synthetic construct
  source 1..17: mol_type = other RNA
gtacattctagatagcc

SEQ ID NO: 43 - RNA, 17 nt, synthetic construct
  source 1..17: mol_type = other RNA
ggctatctagaatgtac

SEQ ID NO: 44 - RNA, 24 nt, synthetic construct
  source 1..24: mol_type = other RNA
ggacatggattcttgtctgtgtcc

SEQ ID NO: 45 - RNA, 24 nt, synthetic construct
  source 1..24: mol_type = other RNA
gatctgtgtcttagacgtgttgcc

SEQ ID NO: 46 - RNA, 30 nt, synthetic construct
  source 1..30: mol_type = other RNA
ccagagtcgctgagattcgtggcgctatat

SEQ ID NO: 47 - RNA, 32 nt, synthetic construct; identical to SEQ ID NO: 3
  source 1..32: mol_type = other RNA

SEQ ID NO: 48 - RNA, 32 nt, synthetic construct; identical to SEQ ID NO: 3
  source 1..32: mol_type = other RNA

SEQ ID NO: 49 - RNA, 32 nt, synthetic construct
  source 1..32: mol_type = other RNA
gactggagttcagacgtgtgctcttccgatct

SEQ ID NO: 50 - RNA, 24 nt, synthetic construct
  source 1..24: mol_type = other RNA
gactggagttcagacgtgtgctct

SEQ ID NO: 51 - RNA, 32 nt, synthetic construct
  source 1..32: mol_type = other RNA
gatcgtgacgactcttgtctgctgtcctgatc

SEQ ID NO: 52 - RNA, 32 nt, synthetic construct
  source 1..32: mol_type = other RNA
cgtctccagcatgtgtaggtctctgtctctga

SEQ ID NO: 53 - RNA, 21 nt, synthetic construct
  source 1..21: mol_type = other RNA
ggagttcagacgtgttgctct

SEQ ID NO: 54 - RNA, 26 nt, synthetic construct
  source 1..26: mol_type = other RNA
ctggagttcgttgctcttccgatctc

SEQ ID NO: 55 - RNA, 25 nt, synthetic construct
  source 1..25: mol_type = other RNA
ctggacagacgtgtcttccgatctc

SEQ ID NO: 56 - RNA, 32 nt, synthetic construct
  source 1..32: mol_type = other RNA
ctggagttcagatcagacgtgtgtgttgctct

SEQ ID NO: 57 - RNA, 32 nt, synthetic construct
  source 1..32: mol_type = other RNA
ctggagttcagacgtgtagctcgtgtgatctc